European Patent Application EP 4 606 902 A1, published August 27, 2025. Title: PREPARATION OF ENANTIO-SPECIFIC EPOXIDES. Applicant: Vilnius University. Application EM. The sequence listing filed with the application follows.

SEQUENCE LISTING (18 sequences)

SEQ ID NO: 1 - protein, 81 aa, Metagenomic sequence
MTDTGTPFDQLPRYVRVRSEPDATFVEFDFAIGYPELFVELVLPRQAFEQFCQHNHVRHMDAAMAQAVDDDMHKWRYGDSQ

SEQ ID NO: 2 - protein, 331 aa, Metagenomic sequence
MNIEIKTTSVEPIRHTFSHTRRRFGDKPASRYQEASFDLESARNFHYRPLWQPDKLLNDPSRTAVVMADWYRVSDPRQFYYGPYVQTRAKMQENAEHDFVFCEKRNLLAGLDPHSREQIARLLLPLRHAEMGANMNNSGIAADGFGTSVTQMHMFHAMDRLAIAQYLSRIGLMLEDDGLALLAQAKQQWLEDPAWQGVRRYVEDSLVIKDWFELTLAQNLVSDGLLYPLLFGKFDEQLSAAGHGQVGMLTEFMRLWFGETQRWVDALVKTVAAESPANRELLERWIATWRGRALEALAPLAAIGPGHEALQAVDNEFGARLKKLGLTGAAA

SEQ ID NO: 3 - protein, 89 aa, Metagenomic sequence
MTSLVYIAFQDNDNARYIVEAITEDNPHAEVQYQPAMIRVQAEQRLEIQRATVEEKIGRTWDVQEMLIDVITLGGNVEEDEDSFTLHWN

SEQ ID NO: 4 - protein, 504 aa, Metagenomic sequence
MAAKRLNQKEKYRCMTRDLGWEPSYQSKEDIFPYERFEGIKITDWDKWEDPFRLTMDAYWKYQAEKEKKLYAILDAFSQNNGHTNISDARYVNALKLFLSGVTPLEYQAYQGFARVGRHFGGAGARVACQMQAIDELRHVQTQIHAMSHYNKHFNGLHDFAHMHDRVWFLSVPKSFFEDARSAGPFEFLTAISFSFEYVLTNLLFVPFMSGAAFNGDMATVTFGFSAQSDEARHMTLGLEVIKFMLEQHEDNVPIIQRWIDKWFWRGYRLLTLVGMMMDYMLPNKVMSWAEAWKVYFEDAGGALFKDLERYGIRPPKYVEQAQIGKDHISHQAWSIFYQYSQATNFHTWMPTDEELDWLSAKYPDTFDAVYRPRYEHWRALQEKGERFYNPSLPMLCQICQIPLAFTEPDDPTTLSHRSHEHEGERYHFCSDGCCEIFQYEPMKYIQAWLPVHQILQGNCGGADVEAVVRDYYNINPGQDNFEYQDSPEHQRWQAWHPQTKAPA

SEQ ID NO: 5 - protein, 119 aa, Metagenomic sequence
MPVTAIGAYSAQPLDSQQHFNGAQLVYLGWDRHLMFCAPFTFPLPPDMAFADFLEQVVKPAIAPHPDARQVNFAEARWRLDGQPFTPELQLSLIANGIAHKSLLNLVTPGLNGLAGSSN

SEQ ID NO: 6 - protein, 353 aa, Metagenomic sequence
MSYLVTIEPTGEQIEVSPGQTILQAALRQGVWLPFACGHGTCATCKVQVLEGEVDIGAASTFALMDMEREEGKILACCAMPTSDLVIEADIDVDPDFQAFPVEDYRAVVSQLVDLSPTIKGVHLKLDRPMAFQAGQYINLQLPGIEGTRAFSLANPPSRADELELHVRLVEGGLVTGHIHQALKVGDGLELSGPYGQFFVRGSQPGGLIFIAGGSGLSSPQSMIVDLLEQGDERPMVLFQGARNRAELYNHGLFEELALRHSNFRYVPALSQAADDEAWQGFRGYVHDAAKQHFDARFSANKAYLCGPPPMIDAAITCLMQGRLFERDIFMERFYSAADGATDGQRSALFKRI

SEQ ID NO: 7 - protein, 97 aa, Metagenomic sequence
MNLPDESLDMQPADLDTRKRFVRVTGSRGSNFVEFDFAIGEPELFVEMILTHEAFDEFCRTNQVESMPALPEVDGEDDEAGQWDWRLADATQVRFKN

SEQ ID NO: 8 - protein, 330 aa, Metagenomic sequence
MHIDLRTVSIQPLRQTFDHLARRFGDKPASRYQEGSYDIQAAENLHYRPTWDPDQALYDAGITKIVMSDWYALKDPRQFYYSTYTLARARQQENTEANFSFVETRGLADMLPDDLRRRALNLLVPLRHAAWGANLNNTFICSYGYGTVFTQPCMYHAMDNLGIAQYLSRIGLLLGGTEALEEGKAAWMDGDAWQGLRRYTEDCLVVRDPLELFVAQNVAMDGLLYPLVYERIVDEQFAANGGSVVAMLAQFMSDWFDETRKWVDAVMKVAAAESEQNREQLQAWTITWRDRAAAALLPVIEQAFAGQADEVMGEQLAAFKARLDKTGVVV

SEQ ID NO: 9 - protein, 89 aa, Metagenomic sequence
MSTVFIALQTNEETRPIIEAIELDNPEAVVNREPAMVKINAPGRLVIRRETIEEQLGRSFDMQELNVNLITLSGNVVEDEDSLTLSWGN

SEQ ID NO: 10 - protein, 506 aa, Metagenomic sequence
MDMKTANKKMNAKDKYRLLTRDLAWDPSYRTEEEIFPYIAYEGLKIHDWNKWEDPFRLTMDAYWKYQAEKERKFYAIIDAHAQNNGHLNITDARYLSALKIFLQAISPAEYSSHKGFARAGREFRGVGTQVACQMQAIDELRHAQTQIHALSNYNKFYNGFHAFADQRDRIWYTSVARSFFDDAMSAGPFEFMIAIGFSFEYVLTNLLFVPFMSGAAYNGDMATVTFGFSAQSDEARHMTLGLECIKFMLEQDPDNLPIVQGWIDKWFWRGFRVLGLVSTMMDYMLPKRVMSWREAWEIYGAENGGALFKDLARYGIRPPKSWDDAEAAIDHMSHQFMLGFYQWSFGTSFHAWIPSDEDLQWLSAKYPTTFDKYYRPRWEHIKKLEAAGTPLKNYGLAKLCQCCQLPCVFTEPDDPTLICHRETEYKGDKYHFCSDHCQSIFENEPEKYIQAWLPMPALFQAPTNGDLGAWMDWVSLKDGQDNGDFADSADRRNFEMWRGMATSNQ

SEQ ID NO: 11 - protein, 118 aa, Metagenomic sequence
MPVVARKEYVGVARDRVENFNGKQLVYVSWDHHLLFAAPFLLCLPPQTRFAELLETALKPLLQADPDAAAVDWQAVQWLKGNQPWVPNFEASLADNGIGHKDQLRFKTPGLNSICAVS

SEQ ID NO: 12 - protein, 352 aa, Metagenomic sequence
MSYELTIEPLGQTIEIEEGQTILDAALRAGIYLPHACCHGLCATCKIQVVDGEIEHGEASSFALMDFEREEKKCLACCATAESDLVIEAEIDEDPDAENLPVRDFAGTVSRIETLTPTIKGVWIKLDGAGMHFQAGQYINLQLPDGIGSRAFSVASAPADGSEIELNIRIVPGGRGTAYVHEQLRVGERVSITGPYGRFFVKKSARTPVIFMGGGSGLSSPRSMILDLLAEGCELPITLIYGQRNRDELYYHEEFLAMARQHANFSYVPALSHEPEDSDWQGFRGFVHDAAKAHFDNDFRGHKAYLCGPPLMIDSCISTLMQGRLFERDIYTEKFISAADAQQVRSPLFKAV

SEQ ID NO: 13 - protein, 95 aa, Metagenomic sequence
MSEKSLGLEPFELDTRRKFVRVTGQRGDKFIEFDFAIGEPELFVEMILTPDAFAEFCEANQVEQMPAVTAQGEDTEDEQWDWRLADATQVRFKTE

SEQ ID NO: 14 - protein, 330 aa, Metagenomic sequence
MQIDLRTVTIEPLRVGYDHLIRRFGNKPASRYQEGSYDLQAAENLHYRPTWDPDQELYDASFSKILMPDWYDLKDPRQFYYNPYTLTRARQQENAEANFKFVETRGLAELLPEQLREAALKLLVPLRHAAWGANQNNTLMCGYGYGAVFTQPCIYHAMDNLGTAQYLSRLGLLLGGTEALDAGKDAWMNDRAWQGLRRYTEDTLVIRDPIELFVAQNLALDGLLYPLVYERIVDDLFAAEGGTAVAMLCQFMREWFDETRKWVDAVIKTMAAESEHNREQLQNWTRHWRDRATAALLPVIEQVLADRADAVMEEQLLAFKARLDKTGLVT

SEQ ID NO: 15 - protein, 89 aa, Metagenomic sequence
MSTVFIALQANEETRPIIEAIELDNPEAVVNREPAMVKINAPGRLVIQRETIEEQMGRSYDMQELNVNLITLSGNVEEDEDSLTLTWAD

SEQ ID NO: 16 - protein, 507 aa, Metagenomic sequence
MDMKTANKKLGAKEKYRLLTRDLAWEPTYRNKEEIFPYIQYEGLKIHDWSKWEDPFRLTMDAYWKYQAEKERKFYAIIDAHAQNNGHLNITDARYLSALKIFLQAISPGEYSAHKGFARVGREFAGAGTQVACQMQAIDEIRHAQTQVHALSNYNKFYNGFHAFAEQRDRIWYTSVARSFFDDAMSAGPFEFMMAIGFSFEYVLTNLLFVPFMSGAAYNGDMATVTFGFSAQSDEARHMTLGLECIKFMLEQDPDNLPIVQGWIDKWFWRGIRVLSLVSTMMDYMLPKRVMSWREAWNIYGAENGGALFRDLARYGIRPPKHWDHAVDAIDHMSHQFMLALYQWKFGTAFHVWVPSDEDMDWLSAKYPDTFDKYYRPRWDYIKQQEAASGAPFNNFGLPKLCQCCQLPTLFTEPGDPTLICHRQSEYKGDVYHFCSDGCKAIFDNEPEKYIQAWLPMPGLMQAPLHGDLGAWMDWAFLKDGQDNGDFATSQDRANFERWRAQSTSNQ

SEQ ID NO: 17 - protein, 118 aa, Metagenomic sequence
MPVVARKEYVGVARDRIENFNGKQLVFVSWDHHLLFAAPMMFCVEPQSTLGELIDNHLMPLLRIDADAAAIDWDKAEWLKGTEPWVPDFSASLEVNGIGHKVQLRFKTPQLNTVCAVR

SEQ ID NO: 18 - protein, 352 aa, Metagenomic sequence
MSYELTIEPLGQTIEIEEGQTILDAALRAGIYLPHACGHGLCATCKVQVVDGEIEHGEASTFALMDFEREEQKCLACCATAESDIVIEAEVDEDPDSLNLPVQDFYGVVSRIESLTPTIKGVWIKLENAGDMQFQAGQYINLMLPDEIGSRAFSIASVPGADELELNIRVVPGGRGTLYVHEQMRVGERVHLTGPYGRLFVKKSADLPVIFMAGGSGLSSPRSMILDLLNEGFARPITLIYGQRNREELYYHDEFLALGEQHGNFTYVPALSHEPEGSDWQGARGFVHEVAKNHFDNDFLEHKAYLCGPPLMIESCIGALMQGRLFERDIYTEKFISAADAQQVHSPLFKAI